European Patent Application EP 4 410 314 A1, published August 7, 2024. Title: Combination Therapy. Applicant: ADC Therapeutics SA. The sequence listing filed with the application follows.

SEQUENCE LISTING (10 sequences)

SEQ ID NO: 1 - protein, 109 aa, synthetic construct
QVQLVQSGAEVKKPGSSVKVSCKASGYTFTSYWLHWVRQAPGQGLEWIGYINPRNDYTEYNQNFKDKATITADESTNTAYMELSSLRSEDTAFYFCARRDITTFYWGQG

SEQ ID NO: 2 - protein, 106 aa, synthetic construct
DIQLTQSPSSLSASVGDRVTMSCKSSQSVLYSANHKNYLAWYQQKPGKAPKLLIYWASTRESGVPSRFSGSGSGTDFTFTISSLQPEDIATYYCHQYLSSWTFGQG

SEQ ID NO: 3 - protein, 445 aa, synthetic construct
QVQLVQSGAEVKKPGSSVKVSCKASGYTFTSYWLHWVRQAPGQGLEWIGYINPRNDYTEYNQNFKDKATITADESTNTAYMELSSLRSEDTAFYFCARRDITTFYWGQGTLVTVSSASTKGPSVFPLAPSSKSTSGGTAALGCLVKDYFPEPVTVSWNSGALTSGVHTFPAVLQSSGLYSLSSVVTVPSSSLGTQTYICNVNHKPSNTKVDKKVEPKSCDKTHTVPPVPAPELLGGPSVFLFPPKPKDTLMISRTPEVTCVVVDVSHEDPEVKFNWYVDGVEVHNAKTKPREEQYNSTYRVVSVLTVLHQDWLNGKEYKCKVSNKALPAPIEKTISKAKGQPREPQVYTLPPSRDELTKNQVSLTCLVKGFYPSDIAVEWESNGQPENNYKTTPPVLDSDGSFFLYSKLTVDKSRWQQGNVFSCSVMHEALHNHYTQKSLSLSPG

SEQ ID NO: 4 - protein, 219 aa, synthetic construct
DIQLTQSPSSLSASVGDRVTMSCKSSQSVLYSANHKNYLAWYQQKPGKAPKLLIYWASTRESGVPSRFSGSGSGTDFTFTISSLQPEDIATYYCHQYLSSWTFGQGTKVEIKRTVAAPSVFIFPPSDEQLKSGTASVVCLLNNFYPREAKVQWKVDNALQSGNSQESVTEQDSKDSTYSLSSTLTLSKADYEKHKVYACEVTHQGLSSPVTKSFNRGES

SEQ ID NO: 5 - protein, 5 aa, Mus musculus
SYWLH

SEQ ID NO: 6 - protein, 17 aa, Mus musculus
YINPRNDYTEYNQNFKD

SEQ ID NO: 7 - protein, 7 aa, Mus musculus
RDITTFY

SEQ ID NO: 8 - protein, 14 aa, Mus musculus
KSSQSVLYSANHKN

SEQ ID NO: 9 - protein, 7 aa, Mus musculus
WASTRES

SEQ ID NO: 10 - protein, 8 aa, Mus musculus
HQYLSSWT